European Patent Application EP 4 756 016 A1, published June 10, 2026. Title: 经改造的萤火虫萤光素酶、其制备方法及应用. Applicant: 上海碧云天生物技术有限公司. Application CN. The sequence listing filed with the application follows.

SEQUENCE LISTING (7 sequences)

SEQ ID NO: 1 - protein, 545 aa, Photuris pensylvanica [sequence omitted]

SEQ ID NO: 2 - protein, 544 aa, synthetic construct
MADKNILYGPEPFYPLEDGTAGEQMFDALSRYAAIPGCIALTNAHTKENVLYEEFLKLSCRLAESFKKYGLKQNDTIAVCSENSLQFFLPVIASLYLGIIVAPVNDKYIERELIHSLGIVKPRIVFCSKNTFQKVLNVKSKLKSIETIIILDLNEDLGGYQCLNNFISQNSDSNLDVKKFKPYSFNRDDQVASIMFSSGTTGLPKGVMLTHKNIVARFSIAKDPTFGNAINPTSAILTVIPFHHGFGMMTTLGYFTCGFRVVLMHTFEEKLFLQSLQDYKVESTLLVPTLMAFLAKSALVEKYDLSHLKEIASGGAPLSKEIGEMVKKRFKLNFVRQGYGLTETTSAVLITPKGDAKPGSTGKIVPLHAVKVVDPTTGKILGPNEPGELYFKGPMIMKGYYNNEEATKAIIDNDGWLRSGDIAYYDNDGHFYIVDRLKSLIKYKGYQVAPAEIEGILLQHPYIVDAGVTGIPDEAAGELPAAGVVVQTGKYLNEQIVQDYVASQVSTAKWLRGGVKFLDEIPKGSTGKIDRKVLRQMLEKHTNG

SEQ ID NO: 3 - DNA, 1632 bp, synthetic construct
  source 1..1632: mol_type = other DNA
atggcagataagaatattttatatgggcccgaaccattttatcccttggaagatgggacggctggagaacagatgtttgacgcattatctcgttatgcagctattccgggctgcatagcattgacaaatgctcatacaaaagaaaatgttttatatgaagagtttctgaaactgtcgtgtcgtttagcggaaagttttaaaaagtatggattaaaacaaaacgacacaatagcggtgtgtagcgaaaatagtctgcaatttttccttcctgtaattgcatcattgtatcttggaataattgtggcacctgttaacgataaatacattgaacgtgaattaatacacagtcttggtattgtaaaaccacgcatagttttttgctccaagaatacttttcaaaaagtactgaatgtaaaatctaaattaaaatctattgaaactattattatattagacttaaatgaagacttaggaggttatcaatgcctcaacaactttatttctcaaaattccgatagtaatctggacgtaaaaaaatttaaaccctattcttttaatcgagacgatcaggttgcgtcgattatgttttcttctggtacaactggtctgccgaagggagtcatgctaactcacaagaatattgttgcacgattttctattgcaaaagatcctacttttggtaacgcaattaatcccacgtcagcaattttaacggtaatacctttccaccatggttttggtatgatgaccacattaggatactttacttgtggattccgagttgttctaatgcacacgtttgaagaaaaactatttctacaatcattacaagattataaagtggaaagtactttacttgtaccaacattaatggcatttcttgcaaaaagtgcattagttgaaaagtacgatttatcgcacttaaaagaaattgcatctggtggcgcacctttatcaaaagaaattggggagatggtgaaaaaacggtttaaattaaactttgtcaggcaagggtatggattaacagaaaccacttcggctgttttaattacaccgaaaggtgacgccaaaccgggatcaactggtaaaatagtaccattacacgctgttaaagttgtcgatcctacaacaggaaaaattttggggccaaatgaacctggagaattgtattttaaaggcccgatgataatgaagggttattataataatgaagaagctactaaagcaattattgataatgacggatggttgcgctctggtgatattgcttattatgacaatgatggccatttttatattgtggacaggctgaagtcactgattaaatataaaggttatcaggttgcacctgctgaaattgagggaatactcttacaacatccgtatattgttgatgccggcgttactggtataccggatgaagccgcgggcgagcttccagctgcaggtgttgtagtacagactggaaaatatctaaacgaacaaatcgtacaagattatgttgccagtcaagtttcaacagccaaatggctacgtggtggggtgaaatttttggatgaaattcccaaaggatcaactggaaaaattgacagaaaagtgttaagacaaatgttagaaaaacacaccaatggg

SEQ ID NO: 4 - protein, 544 aa, synthetic construct
MADKNILYGPEPFYPLEDGTAGEQMFDALSRYAAIPGCIALTNAHTKENVLYEEFLKLSCRLAESFKKYGLKQNDTIAVCSENSLQFFLPVIASLYLGIIVAPVNDKYIERELIHSLGIVKPRIVFCSKNTFQKVLNVKSKLKSIETIIILDLNEDLGGYQCLNNFISQNSDSNLDVKKFKPYSFNRDDQVASIMFSSGTTGLPKGVMLTHKNIVARFSIAKDPTFGNAINPTSAILTVIPFHHGFGMMTTLGYFTCGFRVVLMHTFEEKLFLQSLQDYKVESTLLVPTLMALLAKSALVEKYDLSHLKEIASGGAPLSKEIGEMVKKRFKLNFVRQGYGLTETTSAVLITPKGDAKPGSTGKIVPLHAVKVVDPTTGKILGPNEPGELYFKGPMIMKGYYNNEEATKAIIDNDGWLRSGDIAYYDNDGHFYIVDRLKSLIKYKGYQVAPAEIEGILLQHPYIVDAGVTGIPDEAAGELPAAGVVVQTGKYLNEQIVQDYVASQVSTAKWLRGGVKFLDEIPKGSTGKIDRKVLRQMLEKHTNG

SEQ ID NO: 5 - protein, 544 aa, synthetic construct
MADKNILYGPEPFYPLEDGTAGEQMFDALSRYAAIPGCIALTNAHTKENVLYEEFLKLSCRLAESFKKYGLKQNDTIAVCSENSLQFFLPVIASLYLGIIVAPVNDKYIERELIHSLGIVKPRIVFCSKNTFQKVLNVKSKLKSIETIIILDLNEDLGGYQCLNNFISQNSDSNLDVKKFKPYSFNRDDQVASIMFSSGTTGLPKGVMLTHKNIVARFSIAKDPTFGNAINPTSAILTVIPFHHGFGMMTTLGSFTCGFRVVLMHTFEEKLFLQSLQDYKVESTLLVPTLMAFLAKSALVEKYDLSHLKEIASGGAPLSKEIGEMVKKRFKLNFVRQGYGLTETTSAVLITPKGDAKPGSTGKIVPLHAVKVVDPTTGKILGPNEPGELYFKGPMIMKGYYNNEEATKAIIDNDGWLRSGDIAYYDNDGHFYIVDRLKSLIKYKGYQVAPAEIEGILLQHPYIVDAGVTGIPDEAAGELPAAGVVVQTGKYLNEQIVQDYVASQVSTAKWLRGGVKFLDEIPKGSTGKIDRKVLRQMLEKHTNG

SEQ ID NO: 6 - DNA, 24 bp, synthetic construct
  source 1..24: mol_type = other DNA
gtgctcgagttagtggtgatggtg

SEQ ID NO: 7 - DNA, 29 bp, synthetic construct
  source 1..29: mol_type = other DNA
agatatacatatggcagataagaatattt